European Patent Application EP 4 186 928 A1, published May 31, 2023. Title: FUSION POLYPEPTIDE AND POLYPEPTIDE DIMER, AND USE THEREOF. Applicant: Nanjing Normal University. The sequence listing filed with the application follows.

SEQUENCE LISTING (34 sequences)

SEQ ID NO: 1 - protein, 153 aa, Homo sapiens
MYRMQLLSCIALSLALVTNSAPTSSSTKKTQLQLEHLLLDLQMILNGINNYKNPKLTRMLTFKFYMPKKATELKHLQCLEEELKPLEEVLNLAQSKNFHLRPRDLISNINVIVLELKGSETTFMCEYADETATIVEFLNRWITFCQSIISTLT

SEQ ID NO: 2 - protein, 126 aa, Artificial Sequence
  IL-2-1
RDLISNINVIVLELKGSETTFMCEYADETATIVEFLNRWITFSQSIISTLTGSGPASSSTKKTQLQLEHLLLDLQMILNGINNYKNPKLTRMLTFKFYMPKKATELKHLQCLEEELKPLEEVLNLA

SEQ ID NO: 3 - protein, 135 aa, Artificial Sequence
  IL-2-2
LTRMLTFKFYMPKKATELKHLQCLEEELKPLEEVLNLAQSKNFHLRPRDLISNINVIVLELKGSETTFMCEYADETATIVEFLNRWITFSQSIISTLTGSGPASSSTKKTQLQLEHLLLDLQMILNGINNYKNPK

SEQ ID NO: 4 - protein, 135 aa, Artificial Sequence
  IL-2-3
NPKLTRMLTFKFYMPKKATELKHLQCLEEELKPLEEVLNLAQSKNFHLRPRDLISNINVIVLELKGSETTFMCEYADETATIVEFLNRWITFSQSIISTLTGSGPASSSTKKTQLQLEHLLLDLQMILNGINNYK

SEQ ID NO: 5 - protein, 162 aa, Homo sapiens
MRISKPHLRSISIQCYLCLLLNSHFLTEAGIHVFILGCFSAGLPKTEANWVNVISDLKKIEDLIQSMHIDATLYTESDVHPSCKVTAMKCFLLELQVISLESGDASIHDTVENLIILANNSLSSNGNVTESGCKECEELEEKNIKEFLQSFVHIVQMFINTS

SEQ ID NO: 6 - protein, 118 aa, Artificial Sequence
  IL-15-1
ASIHDTVENLIILANNSLSSNGNVTESGCKECEELEEKNIKEFLQSFVHIVQMFINTSGGGGNWVNVISDLKKIEDLIQSMHIDATLYTESDVHPSCKVTAMKCFLLELQVISLESGD

SEQ ID NO: 7 - protein, 720 aa, Artificial Sequence
  C361-IL2-1
DAHKSEVAHRFKDLGEENFKALVLIAFAQYLQQSPFEDHVKLVNEVTEFAKTCVADESAENCDKSLHTLFGDKLCTVATLRETYGEMADCCAKQEPERNECFLQHKDDNPNLPRLVRPEVDVMCTAFHDNEETFLKKYLYEIARRHPYFYAPELLFFAKRYKAAFTECCQAADKAACLLPKLDELRDEGKASSAKQRLKCASLQKFGERAFKAWAVARLSQRFPKAEFAEVSKLVTDLTKVHTECCHGDLLECADDRADLAKYICENQDSISSKLKECCEKPLLEKSHCIAEVENDEMPADLPSLAADFVESKDVCKNYAEAKDVFLGMFLYEYARRHPDYSVVLLLRLAKTYETTLEKCCEAAAKAEAAARDLISNINVIVLELKGSETTFMCEYADETATIVEFLNRWITFSQSIISTLTGSGPASSSTKKTQLQLEHLLLDLQMILNGINNYKNPKLTRMLTFKFYMPKKATELKHLQCLEEELKPLEEVLNLAGSDPHECYAKVFDEFKPLVEEPQNLIKQNCELFEQLGEYKFQNALLVRYTKKVPQVSTPTLVEVSRNLGKVGSKCCKHPEAKRMPCAEDYLSVVLNQLCVLHEKTPVSDRVTKCCTESLVNRRPCFSALEVDETYVPKEFNAETFTFHADICTLSEKERQIKKQTALVELVKHKPKATKEQLKAVMDDFAAFVEKCCKADDKETCFAEEGKKLVAASQAALGL

SEQ ID NO: 8 - protein, 726 aa, Artificial Sequence
  D56-IL2-2
DAHKSEVAHRFKDLGEENFKALVLIAFAQYLQQSPFEDHVKLVNEVTEFAKTCVADAAAAAKLTRMLTFKFYMPKKATELKHLQCLEEELKPLEEVLNLAQSKNFHLRPRDLISNINVIVLELKGSETTFMCEYADETATIVEFLNRWITFSQSIISTLTGSGPASSSTKKTQLQLEHLLLDLQMILNGINNYKNPKESAENCDKSLHTLFGDKLCTVATLRETYGEMADCCAKQEPERNECFLQHKDDNPNLPRLVRPEVDVMCTAFHDNEETFLKKYLYEIARRHPYFYAPELLFFAKRYKAAFTECCQAADKAACLLPKLDELRDEGKASSAKQRLKCASLQKFGERAFKAWAVARLSQRFPKAEFAEVSKLVTDLTKVHTECCHGDLLECADDRADLAKYICENQDSISSKLKECCEKPLLEKSHCIAEVENDEMPADLPSLAADFVESKDVCKNYAEAKDVFLGMFLYEYARRHPDYSVVLLLRLAKTYETTLEKCCAAADPHECYAKVFDEFKPLVEEPQNLIKQNCELFEQLGEYKFQNALLVRYTKKVPQVSTPTLVEVSRNLGKVGSKCCKHPEAKRMPCAEDYLSVVLNQLCVLHEKTPVSDRVTKCCTESLVNRRPCFSALEVDETYVPKEFNAETFTFHADICTLSEKERQIKKQTALVELVKHKPKATKEQLKAVMDDFAAFVEKCCKADDKETCFAEEGKKLVAASQAALGL

SEQ ID NO: 9 - protein, 721 aa, Artificial Sequence
  A300-IL-2-3
DAHKSEVAHRFKDLGEENFKALVLIAFAQYLQQSPFEDHVKLVNEVTEFAKTCVADESAENCDKSLHTLFGDKLCTVATLRETYGEMADCCAKQEPERNECFLQHKDDNPNLPRLVRPEVDVMCTAFHDNEETFLKKYLYEIARRHPYFYAPELLFFAKRYKAAFTECCQAADKAACLLPKLDELRDEGKASSAKQRLKCASLQKFGERAFKAWAVARLSQRFPKAEFAEVSKLVTDLTKVHTECCHGDLLECADDRADLAKYICENQDSISSKLKECCEKPLLEKSHCIAEVENDEMPANPKLTRMLTFKFYMPKKATELKHLQCLEEELKPLEEVLNLAQSKNFHLRPRDLISNINVIVLELKGSETTFMCEYADETATIVEFLNRWITFSQSIISTLTGSGPASSSTKKTQLQLEHLLLDLQMILNGINNYKGDLPSLAADFVESKDVCKNYAEAKDVFLGMFLYEYARRHPDYSVVLLLRLAKTYETTLEKCCAAADPHECYAKVFDEFKPLVEEPQNLIKQNCELFEQLGEYKFQNALLVRYTKKVPQVSTPTLVEVSRNLGKVGSKCCKHPEAKRMPCAEDYLSVVLNQLCVLHEKTPVSDRVTKCCTESLVNRRPCFSALEVDETYVPKEFNAETFTFHADICTLSEKERQIKKQTALVELVKHKPKATKEQLKAVMDDFAAFVEKCCKADDKETCFAEEGKKLVAASQAALGL

SEQ ID NO: 10 - protein, 720 aa, Artificial Sequence
  A362-IL2-3
DAHKSEVAHRFKDLGEENFKALVLIAFAQYLQQSPFEDHVKLVNEVTEFAKTCVADESAENCDKSLHTLFGDKLCTVATLRETYGEMADCCAKQEPERNECFLQHKDDNPNLPRLVRPEVDVMCTAFHDNEETFLKKYLYEIARRHPYFYAPELLFFAKRYKAAFTECCQAADKAACLLPKLDELRDEGKASSAKQRLKCASLQKFGERAFKAWAVARLSQRFPKAEFAEVSKLVTDLTKVHTECCHGDLLECADDRADLAKYICENQDSISSKLKECCEKPLLEKSHCIAEVENDEMPADLPSLAADFVESKDVCKNYAEAKDVFLGMFLYEYARRHPDYSVVLLLRLAKTYETTLEKCCANPKLTRMLTFKFYMPKKATELKHLQCLEEELKPLEEVLNLAQSKNFHLRPRDLISNINVIVLELKGSETTFMCEYADETATIVEFLNRWITFSQSIISTLTGSGPASSSTKKTQLQLEHLLLDLQMILNGINNYKAADPHECYAKVFDEFKPLVEEPQNLIKQNCELFEQLGEYKFQNALLVRYTKKVPQVSTPTLVEVSRNLGKVGSKCCKHPEAKRMPCAEDYLSVVLNQLCVLHEKTPVSDRVTKCCTESLVNRRPCFSALEVDETYVPKEFNAETFTFHADICTLSEKERQIKKQTALVELVKHKPKATKEQLKAVMDDFAAFVEKCCKADDKETCFAEEGKKLVAASQAALGL

SEQ ID NO: 11 - protein, 726 aa, Artificial Sequence
  C361-IL-2-1-His
DAHKSEVAHRFKDLGEENFKALVLIAFAQYLQQSPFEDHVKLVNEVTEFAKTCVADESAENCDKSLHTLFGDKLCTVATLRETYGEMADCCAKQEPERNECFLQHKDDNPNLPRLVRPEVDVMCTAFHDNEETFLKKYLYEIARRHPYFYAPELLFFAKRYKAAFTECCQAADKAACLLPKLDELRDEGKASSAKQRLKCASLQKFGERAFKAWAVARLSQRFPKAEFAEVSKLVTDLTKVHTECCHGDLLECADDRADLAKYICENQDSISSKLKECCEKPLLEKSHCIAEVENDEMPADLPSLAADFVESKDVCKNYAEAKDVFLGMFLYEYARRHPDYSVVLLLRLAKTYETTLEKCCEAAAKAEAAARDLISNINVIVLELKGSETTFMCEYADETATIVEFLNRWITFSQSIISTLTGSGPASSSTKKTQLQLEHLLLDLQMILNGINNYKNPKLTRMLTFKFYMPKKATELKHLQCLEEELKPLEEVLNLAGSDPHECYAKVFDEFKPLVEEPQNLIKQNCELFEQLGEYKFQNALLVRYTKKVPQVSTPTLVEVSRNLGKVGSKCCKHPEAKRMPCAEDYLSVVLNQLCVLHEKTPVSDRVTKCCTESLVNRRPCFSALEVDETYVPKEFNAETFTFHADICTLSEKERQIKKQTALVELVKHKPKATKEQLKAVMDDFAAFVEKCCKADDKETCFAEEGKKLVAASQAALGLHHHHHH

SEQ ID NO: 12 - protein, 732 aa, Artificial Sequence
  D56-IL-2-2-His
DAHKSEVAHRFKDLGEENFKALVLIAFAQYLQQSPFEDHVKLVNEVTEFAKTCVADAAAAAKLTRMLTFKFYMPKKATELKHLQCLEEELKPLEEVLNLAQSKNFHLRPRDLISNINVIVLELKGSETTFMCEYADETATIVEFLNRWITFSQSIISTLTGSGPASSSTKKTQLQLEHLLLDLQMILNGINNYKNPKESAENCDKSLHTLFGDKLCTVATLRETYGEMADCCAKQEPERNECFLQHKDDNPNLPRLVRPEVDVMCTAFHDNEETFLKKYLYEIARRHPYFYAPELLFFAKRYKAAFTECCQAADKAACLLPKLDELRDEGKASSAKQRLKCASLQKFGERAFKAWAVARLSQRFPKAEFAEVSKLVTDLTKVHTECCHGDLLECADDRADLAKYICENQDSISSKLKECCEKPLLEKSHCIAEVENDEMPADLPSLAADFVESKDVCKNYAEAKDVFLGMFLYEYARRHPDYSVVLLLRLAKTYETTLEKCCAAADPHECYAKVFDEFKPLVEEPQNLIKQNCELFEQLGEYKFQNALLVRYTKKVPQVSTPTLVEVSRNLGKVGSKCCKHPEAKRMPCAEDYLSVVLNQLCVLHEKTPVSDRVTKCCTESLVNRRPCFSALEVDETYVPKEFNAETFTFHADICTLSEKERQIKKQTALVELVKHKPKATKEQLKAVMDDFAAFVEKCCKADDKETCFAEEGKKLVAASQAALGLHHHHHH

SEQ ID NO: 13 - protein, 727 aa, Artificial Sequence
  A300-IL-2-3_His
DAHKSEVAHRFKDLGEENFKALVLIAFAQYLQQSPFEDHVKLVNEVTEFAKTCVADESAENCDKSLHTLFGDKLCTVATLRETYGEMADCCAKQEPERNECFLQHKDDNPNLPRLVRPEVDVMCTAFHDNEETFLKKYLYEIARRHPYFYAPELLFFAKRYKAAFTECCQAADKAACLLPKLDELRDEGKASSAKQRLKCASLQKFGERAFKAWAVARLSQRFPKAEFAEVSKLVTDLTKVHTECCHGDLLECADDRADLAKYICENQDSISSKLKECCEKPLLEKSHCIAEVENDEMPANPKLTRMLTFKFYMPKKATELKHLQCLEEELKPLEEVLNLAQSKNFHLRPRDLISNINVIVLELKGSETTFMCEYADETATIVEFLNRWITFSQSIISTLTGSGPASSSTKKTQLQLEHLLLDLQMILNGINNYKGDLPSLAADFVESKDVCKNYAEAKDVFLGMFLYEYARRHPDYSVVLLLRLAKTYETTLEKCCAAADPHECYAKVFDEFKPLVEEPQNLIKQNCELFEQLGEYKFQNALLVRYTKKVPQVSTPTLVEVSRNLGKVGSKCCKHPEAKRMPCAEDYLSVVLNQLCVLHEKTPVSDRVTKCCTESLVNRRPCFSALEVDETYVPKEFNAETFTFHADICTLSEKERQIKKQTALVELVKHKPKATKEQLKAVMDDFAAFVEKCCKADDKETCFAEEGKKLVAASQAALGLHHHHHH

SEQ ID NO: 14 - protein, 726 aa, Artificial Sequence
  A362-IL-2-3_His
DAHKSEVAHRFKDLGEENFKALVLIAFAQYLQQSPFEDHVKLVNEVTEFAKTCVADESAENCDKSLHTLFGDKLCTVATLRETYGEMADCCAKQEPERNECFLQHKDDNPNLPRLVRPEVDVMCTAFHDNEETFLKKYLYEIARRHPYFYAPELLFFAKRYKAAFTECCQAADKAACLLPKLDELRDEGKASSAKQRLKCASLQKFGERAFKAWAVARLSQRFPKAEFAEVSKLVTDLTKVHTECCHGDLLECADDRADLAKYICENQDSISSKLKECCEKPLLEKSHCIAEVENDEMPADLPSLAADFVESKDVCKNYAEAKDVFLGMFLYEYARRHPDYSVVLLLRLAKTYETTLEKCCANPKLTRMLTFKFYMPKKATELKHLQCLEEELKPLEEVLNLAQSKNFHLRPRDLISNINVIVLELKGSETTFMCEYADETATIVEFLNRWITFSQSIISTLTGSGPASSSTKKTQLQLEHLLLDLQMILNGINNYKAADPHECYAKVFDEFKPLVEEPQNLIKQNCELFEQLGEYKFQNALLVRYTKKVPQVSTPTLVEVSRNLGKVGSKCCKHPEAKRMPCAEDYLSVVLNQLCVLHEKTPVSDRVTKCCTESLVNRRPCFSALEVDETYVPKEFNAETFTFHADICTLSEKERQIKKQTALVELVKHKPKATKEQLKAVMDDFAAFVEKCCKADDKETCFAEEGKKLVAASQAALGLHHHHHH

SEQ ID NO: 15 - protein, 609 aa, Homo sapiens [sequence omitted]

SEQ ID NO: 16 - protein, 4 aa, Artificial Sequence
  linker
GGGG

SEQ ID NO: 17 - protein, 20 aa, Artificial Sequence
  signal peptide
METDTLLLWVLLLWVPGSTG

SEQ ID NO: 18 - protein, 10 aa, Artificial Sequence
  linker
EAAAKAEAAA

SEQ ID NO: 19 - protein, 6 aa, Artificial Sequence
  linker
AAAAAK

SEQ ID NO: 20 - protein, 130 aa, Artificial Sequence
  IL-2*
LTRMLTFKFYMPKKATELKHLQCLEEELKPLEEVLNLAQSKNFHLRPRDLISNINVIVLELKGSETTFMCEYADETATIVEFLNRWITFSQSIISTLTGSGPASSSTKKTQLQLEHLLLDLQMILNGINN

SEQ ID NO: 21 - protein, 135 aa, Artificial Sequence
  circular permulated IL-2
NFHLRPRDLISNINVIVLELKGSETTFMCEYADETATIVEFLNRWITFSQSIISTLTGSGPASSSTKKTQLQLEHLLLDLQMILNGINNYKNPKLTRMLTFKFYMPKKATELKHLQCLEEELKPLEEVLNLAQSK

SEQ ID NO: 22 - protein, 115 aa, Artificial Sequence
  circular permulated IL-15
SIHDTVENLIILANNSLSSNGNVTESGCKECEELEEKNIKEFLQSFVHIVQMFINTSGGGGNWVNVISDLKKIEDLIQSMHIDATLYTESDVHPSCKVTAMKCFLLELQVISLES

SEQ ID NO: 23 - protein, 223 aa, Artificial Sequence
  Fc knob
HTCPPCPAPEAAGGPSVFLFPPKPKDTLMISRTPEVTCVVVDVSHEDPEVKFNWYVDGVEVHNAKTKPREEQYNSTYRVVSVLTVLHQDWLNGKEYKCKVSNKALGAPIEKTISKAKGQPREPQVYTLPPCREEMTKNQVSLWCLVKGFYPSDIAVEWESNGQPENNYKTTPPVLDSDGSFFLYSKLTVDKSRWQQGNVFSCSVMHEALHNHYTQKSLSLSPG

SEQ ID NO: 24 - protein, 223 aa, Artificial Sequence
  Fc hole
HTCPPCPAPEAAGGPSVFLFPPKPKDTLMISRTPEVTCVVVDVSHEDPEVKFNWYVDGVEVHNAKTKPREEQYNSTYRVVSVLTVLHQDWLNGKEYKCKVSNKALGAPIEKTISKAKGQPREPQVCTLPPSREEMTKNQVSLSCAVKGFYPSDIAVEWESNGQPENNYKTTPPVLDSDGSFFLVSKLTVDKSRWQQGNVFSCSVMHEALHNHYTQKSLSLSPG

SEQ ID NO: 25 - protein, 368 aa, Artificial Sequence
  IL-2-knob
HTCPPCPAPEAAGGPSVFLFPPKPKDTLMISRTPEVTCVVVDVSHEDPEVKFNWYVDGVEVHNAKTKPREEQYNSTYRVVSVLTVLHQDWLNGKEYKCKVSNKALGAPIEKTISKAKGQPREPQVYTLPPCREEMTKNQVSLWCLVKGFYPSDIAVEWESNGQPENNYKTTPPVLDSDGSFFLYSKLTVDKSRWQQGNVFSCSVMHEALHNHYTQKSLSLSPGGGGGSGGGGSNFHLRPRDLISNINVIVLELKGSETTFMCEYADETATIVEFLNRWITFSQSIISTLTGSGPASSSTKKTQLQLEHLLLDLQMILNGINNYKNPKLTRMLTFKFYMPKKATELKHLQCLEEELKPLEEVLNLAQSK

SEQ ID NO: 26 - protein, 398 aa, Artificial Sequence
  CD25-hole
HTCPPCPAPEAAGGPSVFLFPPKPKDTLMISRTPEVTCVVVDVSHEDPEVKFNWYVDGVEVHNAKTKPREEQYNSTYRVVSVLTVLHQDWLNGKEYKCKVSNKALGAPIEKTISKAKGQPREPQVCTLPPSREEMTKNQVSLSCAVKGFYPSDIAVEWESNGQPENNYKTTPPVLDSDGSFFLVSKLTVDKSRWQQGNVFSCSVMHEALHNHYTQKSLSLSPGGGGGSGGGGSELCDDDPPEIPHATFKAMAYKEGTMLNCECKRGFRRIKSGSLYMLCTGNSSHSSWDNQCQCTSSATRNTTKQVTPQPEEQKERKTTEMQSPMQPVDQASLPGHCREPPPWENEATERIYHFVVGQMVYYQCVQGYRALHRGPAESVCKMTHGKTRWTQPQLICTG

SEQ ID NO: 27 - protein, 368 aa, Artificial Sequence
  IL-2-hole
HTCPPCPAPEAAGGPSVFLFPPKPKDTLMISRTPEVTCVVVDVSHEDPEVKFNWYVDGVEVHNAKTKPREEQYNSTYRVVSVLTVLHQDWLNGKEYKCKVSNKALGAPIEKTISKAKGQPREPQVCTLPPSREEMTKNQVSLSCAVKGFYPSDIAVEWESNGQPENNYKTTPPVLDSDGSFFLVSKLTVDKSRWQQGNVFSCSVMHEALHNHYTQKSLSLSPGGGGGSGGGGSNFHLRPRDLISNINVIVLELKGSETTFMCEYADETATIVEFLNRWITFSQSIISTLTGSGPASSSTKKTQLQLEHLLLDLQMILNGINNYKNPKLTRMLTFKFYMPKKATELKHLQCLEEELKPLEEVLNLAQSK

SEQ ID NO: 28 - protein, 398 aa, Artificial Sequence
  CD25-knob
HTCPPCPAPEAAGGPSVFLFPPKPKDTLMISRTPEVTCVVVDVSHEDPEVKFNWYVDGVEVHNAKTKPREEQYNSTYRVVSVLTVLHQDWLNGKEYKCKVSNKALGAPIEKTISKAKGQPREPQVYTLPPCREEMTKNQVSLWCLVKGFYPSDIAVEWESNGQPENNYKTTPPVLDSDGSFFLYSKLTVDKSRWQQGNVFSCSVMHEALHNHYTQKSLSLSPGGGGGSGGGGSELCDDDPPEIPHATFKAMAYKEGTMLNCECKRGFRRIKSGSLYMLCTGNSSHSSWDNQCQCTSSATRNTTKQVTPQPEEQKERKTTEMQSPMQPVDQASLPGHCREPPPWENEATERIYHFVVGQMVYYQCVQGYRALHRGPAESVCKMTHGKTRWTQPQLICTG

SEQ ID NO: 29 - protein, 165 aa, Artificial Sequence
  CD25ecd
ELCDDDPPEIPHATFKAMAYKEGTMLNCECKRGFRRIKSGSLYMLCTGNSSHSSWDNQCQCTSSATRNTTKQVTPQPEEQKERKTTEMQSPMQPVDQASLPGHCREPPPWENEATERIYHFVVGQMVYYQCVQGYRALHRGPAESVCKMTHGKTRWTQPQLICTG

SEQ ID NO: 30 - protein, 10 aa, Artificial Sequence
  linker
GGGGSGGGGS

SEQ ID NO: 31 - protein, 373 aa, Artificial Sequence
  IL-2-knob-full
HHHHHHTCPPCPAPEAAGGPSVFLFPPKPKDTLMISRTPEVTCVVVDVSHEDPEVKFNWYVDGVEVHNAKTKPREEQYNSTYRVVSVLTVLHQDWLNGKEYKCKVSNKALGAPIEKTISKAKGQPREPQVYTLPPCREEMTKNQVSLWCLVKGFYPSDIAVEWESNGQPENNYKTTPPVLDSDGSFFLYSKLTVDKSRWQQGNVFSCSVMHEALHNHYTQKSLSLSPGGGGGSGGGGSNFHLRPRDLISNINVIVLELKGSETTFMCEYADETATIVEFLNRWITFSQSIISTLTGSGPASSSTKKTQLQLEHLLLDLQMILNGINNYKNPKLTRMLTFKFYMPKKATELKHLQCLEEELKPLEEVLNLAQSK

SEQ ID NO: 32 - protein, 406 aa, Artificial Sequence
  CD25-hole-full
HTCPPCPAPEAAGGPSVFLFPPKPKDTLMISRTPEVTCVVVDVSHEDPEVKFNWYVDGVEVHNAKTKPREEQYNSTYRVVSVLTVLHQDWLNGKEYKCKVSNKALGAPIEKTISKAKGQPREPQVCTLPPSREEMTKNQVSLSCAVKGFYPSDIAVEWESNGQPENNYKTTPPVLDSDGSFFLVSKLTVDKSRWQQGNVFSCSVMHEALHNHYTQKSLSLSPGGGGGSGGGGSELCDDDPPEIPHATFKAMAYKEGTMLNCECKRGFRRIKSGSLYMLCTGNSSHSSWDNQCQCTSSATRNTTKQVTPQPEEQKERKTTEMQSPMQPVDQASLPGHCREPPPWENEATERIYHFVVGQMVYYQCVQGYRALHRGPAESVCKMTHGKTRWTQPQLICTGDYKDDDDK

SEQ ID NO: 33 - protein, 373 aa, Artificial Sequence
  IL-2-hole-full
HHHHHHTCPPCPAPEAAGGPSVFLFPPKPKDTLMISRTPEVTCVVVDVSHEDPEVKFNWYVDGVEVHNAKTKPREEQYNSTYRVVSVLTVLHQDWLNGKEYKCKVSNKALGAPIEKTISKAKGQPREPQVCTLPPSREEMTKNQVSLSCAVKGFYPSDIAVEWESNGQPENNYKTTPPVLDSDGSFFLVSKLTVDKSRWQQGNVFSCSVMHEALHNHYTQKSLSLSPGGGGGSGGGGSNFHLRPRDLISNINVIVLELKGSETTFMCEYADETATIVEFLNRWITFSQSIISTLTGSGPASSSTKKTQLQLEHLLLDLQMILNGINNYKNPKLTRMLTFKFYMPKKATELKHLQCLEEELKPLEEVLNLAQSK

SEQ ID NO: 34 - protein, 406 aa, Artificial Sequence
  CD25-knob-full
HTCPPCPAPEAAGGPSVFLFPPKPKDTLMISRTPEVTCVVVDVSHEDPEVKFNWYVDGVEVHNAKTKPREEQYNSTYRVVSVLTVLHQDWLNGKEYKCKVSNKALGAPIEKTISKAKGQPREPQVYTLPPCREEMTKNQVSLWCLVKGFYPSDIAVEWESNGQPENNYKTTPPVLDSDGSFFLYSKLTVDKSRWQQGNVFSCSVMHEALHNHYTQKSLSLSPGGGGGSGGGGSELCDDDPPEIPHATFKAMAYKEGTMLNCECKRGFRRIKSGSLYMLCTGNSSHSSWDNQCQCTSSATRNTTKQVTPQPEEQKERKTTEMQSPMQPVDQASLPGHCREPPPWENEATERIYHFVVGQMVYYQCVQGYRALHRGPAESVCKMTHGKTRWTQPQLICTGDYKDDDDK